European Patent Application EP 4 268 848 A2, published November 1, 2023. Title: MONOSPECIFIC PROTEINS WITH IMMUNE CHECKPOINT REGULATION FOR CANCER THERAPY. Applicant: AP Biosciences, Inc. Application EP. The sequence listing filed with the application follows.

SEQUENCE LISTING (43 sequences)

SEQ ID NO: 1 - protein, 217 aa, Homo sapiens
QSVLTQPPSASGTPGQRVTISCSGSSSNIGSNTVNWYQQLPGTAPKLLIYSNNQRPSGVPDRFSGSKSGTSASLAISGLQSEDEADYYCATWDDSLNAWVVFGGGTKLTVLGQPKAAPSVTLFPPSSEELQANKATLVCLISDFYPGAVTVAWKADSSPVKAGVETTTPSKQSNNKYAASSYLSLTPEQWKSHRSYSCQVTHEGSTVEKTVAPTECS

SEQ ID NO: 2 - protein, 118 aa, Homo sapiens
QVQLVQSGAEVKKPGSSVKVSCKASGGTFRRYSISWVRQAPGQGLEWMGGIIPVFGAAKYAQKFQGRVTITADEFTSTAYMELSSLTSEDTAVYYCALSGDSDAFDIWGQGTMVTVSS

SEQ ID NO: 3 - protein, 216 aa, Homo sapiens
QSALTQPASVSGSPGQSITISCTGTSNDVGSYNSVSWYQQHPGKAPKLVIYEVANRPSGVPDRFSGSKSGNTASLTISGLQAEDEADYYCSSYTSSSTLVFGGGTKLTVLGQPKAAPSVTLFPPSSEELQANKATLVCLISDFYPGAVTVAWKADSSPVKAGVETTTPSKQSNNKYAASSYLSLTPEQWKSHRSYSCQVTHEGSTVEKTVAPTECS

SEQ ID NO: 4 - protein, 121 aa, Homo sapiens
QVQLVQSGAKVKKPGSSVKVSCKASGGTFSSYAISWVRQAPGQGLEWMGRIIPILGIANYAQKFQGRVTITADKSTSTAYMELSSLRSEDTAVYYCARVVPGYSYGPFDYWGQGTTVTVSS

SEQ ID NO: 5 - protein, 214 aa, Homo sapiens
SYVLTQPPSVSVTPGKTARIACGGNNLESKIVSWYQQKPGQAPVLVIFYDTDRPSGISERFSGSNSGNTATLTISRVEAGDEADYYCQVWDSNSDHVIFGGGTKLTVLGQPKAAPSVTLFPPSSEELQANKATLVCLISDFYPGAVTVAWKADSSPVKAGVETTTPSKQSNNKYAASSYLSLTPEQWKSHRSYSCQVTHEGSTVEKTVAPTECS

SEQ ID NO: 6 - protein, 126 aa, Homo sapiens
EVQLVESGGVVVQPGGSLRLSCAASGFTFDDYTMHWVRQAPGKGLEWVSLISWDGGSTYYADSVKGRFTISRDNSKNSLYLQMNSLRTEDTALYYCASIYDPPPGSRSALDAFDIWGQGTMVTVSS

SEQ ID NO: 7 - protein, 214 aa, Homo sapiens
SYVLTQPPSVSVTPGKTARIACGGNNLESKIVSWYQQKPGQAPVLVIFYDTDRPSGISERFSGSNSGNTATLTISRVEAGDEADYYCQVWDSNSDHVIFGGGTKLTVLGQPKAAPSVTLFPPSSEELQANKATLVCLISDFYPGAVTVAWKADSSPVKAGVETTTPSKQSNNKYAASSYLSLTPEQWKSHRSYSCQVTHEGSTVEKTVAPAECS

SEQ ID NO: 8 - protein, 118 aa, Homo sapiens
EVQLVESGGGLVKPGGSLRLSCAASGFTFSSYSMNWVRQAPGKGLEWVSSISSSSRYIYYADSVKGRFTISRDNAKNSLYLQMNSLRAEDTAVYYCARQNEDVAFGIWGQGTMVTVSS

SEQ ID NO: 9 - protein, 327 aa, Homo sapiens
ASTKGPSVFPLAPCSRSTSESTAALGCLVKDYFPEPVTVSWNSGALTSGVHTFPAVLQSSGLYSLSSVVTVPSSSLGTKTYTCNVDHKPSNTKVDKRVESKYGPPCPPCPAPEFLGGPSVFLFPPKPKDTLMISRTPEVTCVVVDVSQEDPEVQFNWYVDGVEVHNAKTKPREEQFNSTYRVVSVLTVLHQDWLNGKEYKCKVSNKGLPSSIEKTISKAKGQPREPQVYTLPPSQEEMTKNQVSLTCLVKGFYPSDIAVEWESNGQPENNYKTTPPVLDSDGSFFLYSRLTVDKSRWQEGNVFSCSVMHEALHNHYTQKSLSLSLGK

SEQ ID NO: 10 - protein, 246 aa, synthetic construct
  REGION 1..246: note = OX40 scFv (Clone A4)
QSALTQPPSASGSPGQSVTISCTGTSSDVGGYNYVSWYQQHPGKAPKLMIYEVSQRPSGVPDRFSGSKSGNTASLTVSGLQAEDEADYYCSSYAGSNNLGVFGGGTKLTVSSGGGGSGGGGSGGGGSQVQLVESGGGLVQPGGSLRLSCAASGFTFSSYEMNWVRQAPGKGLEWVSYISSSGSTIYYADSVKGRFTISRDNAKNSLYLQMNSLRAEDTAVYYCARGGVGDAFDIWGQGTMVTVSSA

SEQ ID NO: 11 - protein, 250 aa, synthetic construct
  REGION 1..250: note = OX40 scFv (Clone B17)
YVLTQPPSVSVTPGKTARIACGGNNLESKIVSWYQQKPGQAPVLVIFYDTDRPSGISERFSGSNSGNTATLTISRVEAGDEADYYCQVWDSNSDHVIFGGGTKLTVSSGGGGSGGGGSGGGGSEVQLVESGGVVVQPGGSLRLSCAASGFTFDDYTMHWVRQAPGKGLEWVSLISWDGGSTYYADSVKGRFTISRDNSKNSLYLQMNSLRTEDTALYYCASIYDPPPGSRSALDAFDIWGQGTMVTVSSA

SEQ ID NO: 12 - protein, 243 aa, synthetic construct
  REGION 1..243: note = OX40 scFv (Clone B19)
SYVLTQPPSVSVTPGKTARIACGGNNLESKIVSWYQQKPGQAPVLVIFYDTDRPSGISERFSGSNSGNTATLTISRVEAGDEADYYCQVWDSNSDHVIFGGGTKLTVSSGGGGSGGGGSGGGGSEVQLVESGGGLVKPGGSLRLSCAASGFTFSSYSMNWVRQAPGKGLEWVSSISSSSRYIYYADSVKGRFTISRDNAKNSLYLQMNSLRAEDTAVYYCARQNEDVAFGIWGQGTMVTVSSA

SEQ ID NO: 13 - protein, 241 aa, synthetic construct
  REGION 1..241: note = OX40 scFv (Clone B120)
SYELTQPPSVSVSPGQTASITCSGDTLGDKYASWYQQKPGRSPVLVIYQDSERPSGIPERFSGSNSGNTATLTISGTQAMDEADYYCQAWDSSTSYVFGTGTKVTVSSGGGGSGGGGSGGGGSQVQLQQWGAGLLKPSETLSLTCAVYGGSFSGYYWSWIRQPPGKGLEWIGEINHSGSTNYNPSLKSRVTISVDTSKNQFSLKLSSVTAADTAVYYCARGRWGGSFIYWGQGTLVTVSSA

SEQ ID NO: 14 - protein, 10 aa, synthetic construct
  REGION 1..10: note = peptide linker
GGGGSGGGGS

SEQ ID NO: 15 - protein, 20 aa, synthetic construct
  REGION 1..20: note = signal peptide
METDTLLLWVLLLWVPGSTG

SEQ ID NO: 16 - protein, 704 aa, synthetic construct
  REGION 1..704: note = Anti-PD-L1-clone 6 Heavy Chain-OX40 clone B17 scFv antibody
QVQLVQSGAEVKKPGSSVKVSCKASGGTFRRYSISWVRQAPGQGLEWMGGIIPVFGAAKYAQKFQGRVTITADEFTSTAYMELSSLTSEDTAVYYCALSGDSDAFDIWGQGTMVTVSSASTKGPSVFPLAPCSRSTSESTAALGCLVKDYFPEPVTVSWNSGALTSGVHTFPAVLQSSGLYSLSSVVTVPSSSLGTKTYTCNVDHKPSNTKVDKRVESKYGPPCPPCPAPEFLGGPSVFLFPPKPKDTLMISRTPEVTCVVVDVSQEDPEVQFNWYVDGVEVHNAKTKPREEQFNSTYRVVSVLTVLHQDWLNGKEYKCKVSNKGLPSSIEKTISKAKGQPREPQVYTLPPSQEEMTKNQVSLTCLVKGFYPSDIAVEWESNGQPENNYKTTPPVLDSDGSFFLYSRLTVDKSRWQEGNVFSCSVMHEALHNHYTQKSLSLSLGGGGGSGGGGSYVLTQPPSVSVTPGKTARIACGGNNLESKIVSWYQQKPGQAPVLVIFYDTDRPSGISERFSGSNSGNTATLTISRVEAGDEADYYCQVWDSNSDHVIFGGGTKLTVSSGGGGSGGGGSGGGGSEVQLVESGGVVVQPGGSLRLSCAASGFTFDDYTMHWVRQAPGKGLEWVSLISWDGGSTYYADSVKGRFTISRDNSKNSLYLQMNSLRTEDTALYYCASIYDPPPGSRSALDAFDIWGQGTMVTVSSA

SEQ ID NO: 17 - protein, 696 aa, synthetic construct
  REGION 1..696: note = Anti-PD-L1-clone 6 Heavy Chain-OX40 clone B19 scFv antibody
QVQLVQSGAEVKKPGSSVKVSCKASGGTFRRYSISWVRQAPGQGLEWMGGIIPVFGAAKYAQKFQGRVTITADEFTSTAYMELSSLTSEDTAVYYCALSGDSDAFDIWGQGTMVTVSSASTKGPSVFPLAPCSRSTSESTAALGCLVKDYFPEPVTVSWNSGALTSGVHTFPAVLQSSGLYSLSSVVTVPSSSLGTKTYTCNVDHKPSNTKVDKRVESKYGPPCPPCPAPEFLGGPSVFLFPPKPKDTLMISRTPEVTCVVVDVSQEDPEVQFNWYVDGVEVHNAKTKPREEQFNSTYRVVSVLTVLHQDWLNGKEYKCKVSNKGLPSSIEKTISKAKGQPREPQVYTLPPSQEEMTKNQVSLTCLVKGFYPSDIAVEWESNGQPENNYKTTPPVLDSDGSFFLYSRLTVDKSRWQEGNVFSCSVMHEALHNHYTQKSLSLSLGGGGGSGGGGSYVLTQPPSVSVTPGKTARIACGGNNLESKIVSWYQQKPGQAPVLVIFYDTDRPSGISERFSGSNSGNTATLTISRVEAGDEADYYCQVWDSNSDHVIFGGGTKLTVSSGGGGSGGGGSGGGGSEVQLVESGGGLVKPGGSLRLSCAASGFTFSSYSMNWVRQAPGKGLEWVSSISSSSRYIYYADSVKGRFTISRDNAKNSLYLQMNSLRAEDTAVYYCARQNEDVAFGIWGQGTMVTVSSA

SEQ ID NO: 18 - protein, 707 aa, synthetic construct
  REGION 1..707: note = Anti-PD-L1-OX40 Ab-V1
QVQLVQSGAEVKKPGSSVKVSCKASGGTFRRYSISWVRQAPGQGLEWMGGIIPVFGAAKYAQKFQGRVTITADEFTSTAYMELSSLTSEDTAVYYCALSGDSDAFDIWGQGTMVTVSSASTKGPSVFPLAPCSRSTSESTAALGCLVKDYFPEPVTVSWNSGALTSGVHTFPAVLQSSGLYSLSSVVTVPSSSLGTKTYTCNVDHKPSNTKVDKRVESKYGPPCPPCPAPEFLGGPSVFLFPPKPKDTLMISRTPEVTCVVVDVSQEDPEVQFNWYVDGVEVHNAKTKPREEQFNSTYRVVSVLTVLHQDWLNGKEYKCKVSNKGLPSSIEKTISKAKGQPREPQVYTLPPSQEEMTKNQVSLTCLVKGFYPSDIAVEWESNGQPENNYKTTPPVLDSDGSFFLYSRLTVDKSRWQEGNVFSCSVMHEALHNHYTQKSLSLSLGGGGGSGGGGSYVLTQPPSVSVTPGKTARIACGGNNLESKIVSWYQQKPGQAPVLVIFYDTDRPSGISERFSGSNSGNTATLTISRVEAGDEADYYCQVWDSNSDHVIFGGGTKLTVLSSGGGGSGGGGGGSSRSSLEVQLVESGGVVVQPGGSLRLSCAASGFTFDDYTMHWVRQAPGKGLEWVSLISWDGGSTYYADSVKGRFTISRDNSKNSLYLQMNSLRTEDTALYYCASIYDPPPGSRSALDAFDIWGQGTMVTVSSA

SEQ ID NO: 19 - protein, 708 aa, synthetic construct
  REGION 1..708: note = Anti-PD-L1-OX40 Ab-V2
QVQLVQSGAEVKKPGSSVKVSCKASGGTFRRYSISWVRQAPGQGLEWMGGIIPVFGAAKYAQKFQGRVTITADEFTSTAYMELSSLTSEDTAVYYCALSGDSDAFDIWGQGTMVTVSSASTKGPSVFPLAPCSRSTSESTAALGCLVKDYFPEPVTVSWNSGALTSGVHTFPAVLQSSGLYSLSSVVTVPSSSLGTKTYTCNVDHKPSNTKVDKRVESKYGPPCPPCPAPEFLGGPSVFLFPPKPKDTLMISRTPEVTCVVVDVSQEDPEVQFNWYVDGVEVHNAKTKPREEQFNSTYRVVSVLTVLHQDWLNGKEYKCKVSNKGLPSSIEKTISKAKGQPREPQVYTLPPSQEEMTKNQVSLTCLVKGFYPSDIAVEWESNGQPENNYKTTPPVLDSDGSFFLYSRLTVDKSRWQEGNVFSCSVMHEALHNHYTQKSLSLSLGGGGGSGGGGSYVLTQPPSVSVTPGKTARIACGGNNLESKIVSWYQQKPGQAPVLVIFYDTDRPSGISERFSGSNSGNTATLTISRVEAGDEADYYCQVWDSNSDHVIFGGGTKLTVLGGKGSGGKGTGGKGSGGKGSEVQLVESGGVVVQPGGSLRLSCAASGFTFDDYTMHWVRQAPGKGLEWVSLISWDGGSTYYADSVKGRFTISRDNSKNSLYLQMNSLRTEDTALYYCASIYDPPPGSRSALDAFDIWGQGTMVTVSSA

SEQ ID NO: 20 - protein, 701 aa, synthetic construct
  REGION 1..701: note = Anti-PD-L1-OX40 Ab-V3
QVQLVQSGAEVKKPGSSVKVSCKASGGTFRRYSISWVRQAPGQGLEWMGGIIPVFGAAKYAQKFQGRVTITADEFTSTAYMELSSLTSEDTAVYYCALSGDSDAFDIWGQGTMVTVSSASTKGPSVFPLAPCSRSTSESTAALGCLVKDYFPEPVTVSWNSGALTSGVHTFPAVLQSSGLYSLSSVVTVPSSSLGTKTYTCNVDHKPSNTKVDKRVESKYGPPCPPCPAPEFLGGPSVFLFPPKPKDTLMISRTPEVTCVVVDVSQEDPEVQFNWYVDGVEVHNAKTKPREEQFNSTYRVVSVLTVLHQDWLNGKEYKCKVSNKGLPSSIEKTISKAKGQPREPQVYTLPPSQEEMTKNQVSLTCLVKGFYPSDIAVEWESNGQPENNYKTTPPVLDSDGSFFLYSRLTVDKSRWQEGNVFSCSVMHEALHNHYTQKSLSLSLGGGGGSGGGGSYVLTQPPSVSVTPGKTARIACGGNNLESKIVSWYQQKPGQAPVLVIFYDTDRPSGISERFSGSNSGNTATLTISRVEAGDEADYYCQVWDSNSDHVIFGGGTKLTVLGSASAPTLFPLVSEVQLVESGGVVVQPGGSLRLSCAASGFTFDDYTMHWVRQAPGKGLEWVSLISWDGGSTYYADSVKGRFTISRDNSKNSLYLQMNSLRTEDTALYYCASIYDPPPGSRSALDAFDIWGQGTMVTVSSA

SEQ ID NO: 21 - protein, 706 aa, synthetic construct
  REGION 1..706: note = Anti-PD-L1-OX40 Ab-V4
QVQLVQSGAEVKKPGSSVKVSCKASGGTFRRYSISWVRQAPGQGLEWMGGIIPVFGAAKYAQKFQGRVTITADEFTSTAYMELSSLTSEDTAVYYCALSGDSDAFDIWGQGTMVTVSSASTKGPSVFPLAPCSRSTSESTAALGCLVKDYFPEPVTVSWNSGALTSGVHTFPAVLQSSGLYSLSSVVTVPSSSLGTKTYTCNVDHKPSNTKVDKRVESKYGPPCPPCPAPEFLGGPSVFLFPPKPKDTLMISRTPEVTCVVVDVSQEDPEVQFNWYVDGVEVHNAKTKPREEQFNSTYRVVSVLTVLHQDWLNGKEYKCKVSNKGLPSSIEKTISKAKGQPREPQVYTLPPSQEEMTKNQVSLTCLVKGFYPSDIAVEWESNGQPENNYKTTPPVLDSDGSFFLYSRLTVDKSRWQEGNVFSCSVMHEALHNHYTQKSLSLSLGGGGGSGGGGSYVLTQPPSVSVTPGKTARIACGGNNLESKIVSWYQQKPGQAPVLVIFYDTDRPSGISERFSGSNSGNTATLTISRVEAGDEADYYCQVWDSNSDHVIFGGGTKLTVLGSTSGSGKPGSGEGSTKGEVQLVESGGVVVQPGGSLRLSCAASGFTFDDYTMHWVRQAPGKGLEWVSLISWDGGSTYYADSVKGRFTISRDNSKNSLYLQMNSLRTEDTALYYCASIYDPPPGSRSALDAFDIWGQGTMVTVSSA

SEQ ID NO: 22 - protein, 706 aa, synthetic construct
  REGION 1..706: note = Anti-PD-L1-OX40 Ab-V5
QVQLVQSGAEVKKPGSSVKVSCKASGGTFRRYSISWVRQAPGQGLEWMGGIIPVFGAAKYAQKFQGRVTITADEFTSTAYMELSSLTSEDTAVYYCALSGDSDAFDIWGQGTMVTVSSASTKGPSVFPLAPCSRSTSESTAALGCLVKDYFPEPVTVSWNSGALTSGVHTFPAVLQSSGLYSLSSVVTVPSSSLGTKTYTCNVDHKPSNTKVDKRVESKYGPPCPPCPAPEFLGGPSVFLFPPKPKDTLMISRTPEVTCVVVDVSQEDPEVQFNWYVDGVEVHNAKTKPREEQFNSTYRVVSVLTVLHQDWLNGKEYKCKVSNKGLPSSIEKTISKAKGQPREPQVYTLPPSQEEMTKNQVSLTCLVKGFYPSDIAVEWESNGQPENNYKTTPPVLDSDGSFFLYSRLTVDKSRWQEGNVFSCSVMHEALHNHYTQKSLSLSLGGGGGSGGGGSYELTQPPSVSVTPGQTARIACGGNNLESKIVSWYQQKPGQAPVLVIFYDTDRPSGISERFSGSNSGNTATLTISRVEAGDEADYYCQVWDSNSDHVIFGGGTKLTVLGSTSGSGKPGSGEGSTKGEVQLVESGGVVVQPGGSLRLSCAASGFTFDDYTMHWVRQAPGKGLEWVSLISWDGGSTYYADSVKGRFTISRDNSKNSLYLQMNSLRTEDTALYYCASIYDPPPGSRSALDAFDIWGQGTMVTVSSA

SEQ ID NO: 23 - protein, 706 aa, synthetic construct
  REGION 1..706: note = Anti-PD-L1-OX40 Ab-V6
QVQLVQSGAEVKKPGSSVKVSCKASGGTFRRYSISWVRQAPGQGLEWMGGIIPVFGAAKYAQKFQGRVTITADEFTSTAYMELSSLTSEDTAVYYCALSGDSDAFDIWGQGTMVTVSSASTKGPSVFPLAPCSRSTSESTAALGCLVKDYFPEPVTVSWNSGALTSGVHTFPAVLQSSGLYSLSSVVTVPSSSLGTKTYTCNVDHKPSNTKVDKRVESKYGPPCPPCPAPEFLGGPSVFLFPPKPKDTLMISRTPEVTCVVVDVSQEDPEVQFNWYVDGVEVHNAKTKPREEQFNSTYRVVSVLTVLHQDWLNGKEYKCKVSNKGLPSSIEKTISKAKGQPREPQVYTLPPSQEEMTKNQVSLTCLVKGFYPSDIAVEWESNGQPENNYKTTPPVLDSDGSFFLYSRLTVDKSRWQEGNVFSCSVMHEALHNHYTQKSLSLSLGGGGGSGGGGSYVLTQPPSVSVTPGETARIACGGNNLESKIVSWYQQKPGQAPVLVIFYDTDRPSGISERFSGSNSGNTATLTISRVEAGDEADYYCQVWDSNSDHVVFGGGTKLTVLGSTSGSGKPGSGEGSTKGEVQLVESGGGVVQPGGSLRLSCAASGFTFDDYTMHWVRQAPGKGLEWVSLISWDGGSTYYADSVKGRFTISRDNSKNSLYLQMNSLRTEDTALYYCASIYDPPPGSRSALDAFDIWGQGTMVTVSSA

SEQ ID NO: 24 - protein, 706 aa, synthetic construct
  REGION 1..706: note = Anti-PD-L1-OX40 Ab-V7
QVQLVQSGAEVKKPGSSVKVSCKASGGTFRRYSISWVRQAPGQGLEWMGGIIPVFGAAKYAQKFQGRVTITADEFTSTAYMELSSLTSEDTAVYYCALSGDSDAFDIWGQGTMVTVSSASTKGPSVFPLAPCSRSTSESTAALGCLVKDYFPEPVTVSWNSGALTSGVHTFPAVLQSSGLYSLSSVVTVPSSSLGTKTYTCNVDHKPSNTKVDKRVESKYGPPCPPCPAPEFLGGPSVFLFPPKPKDTLMISRTPEVTCVVVDVSQEDPEVQFNWYVDGVEVHNAKTKPREEQFNSTYRVVSVLTVLHQDWLNGKEYKCKVSNKGLPSSIEKTISKAKGQPREPQVYTLPPSQEEMTKNQVSLTCLVKGFYPSDIAVEWESNGQPENNYKTTPPVLDSDGSFFLYSRLTVDKSRWQEGNVFSCSVMHEALHNHYTQKSLSLSLGGGGGSGGGGSYVLTQPPSVSVTPGQTARIACGGNNLESKIVSWYQQKPGQAPVLVIFYDTDRPSGISERFSGSNSGNTATLTISRVEAGDEADYYCQVWDSNSDHVVFGGGTKLTVLGSTSGSGKPGSGEGSTKGEVQLVESGGGVVQPGGSLRLSCAASGFTFDDYTMHWVRQAPGKGLEWVSLISWDGGSTYYADSVKGRFTISRDNSKNSLYLQMNSLRTEDTALYYCASIYDPPPGSRSALDAFDIWGQGTMVTVSSA

SEQ ID NO: 25 - protein, 706 aa, synthetic construct
  REGION 1..706: note = Anti-PD-L1-OX40 Ab-V8
QVQLVQSGAEVKKPGSSVKVSCKASGGTFRRYSISWVRQAPGQGLEWMGGIIPVFGAAKYAQKFQGRVTITADEFTSTAYMELSSLTSEDTAVYYCALSGDSDAFDIWGQGTMVTVSSASTKGPSVFPLAPCSRSTSESTAALGCLVKDYFPEPVTVSWNSGALTSGVHTFPAVLQSSGLYSLSSVVTVPSSSLGTKTYTCNVDHKPSNTKVDKRVESKYGPPCPPCPAPEFLGGPSVFLFPPKPKDTLMISRTPEVTCVVVDVSQEDPEVQFNWYVDGVEVHNAKTKPREEQFNSTYRVVSVLTVLHQDWLNGKEYKCKVSNKGLPSSIEKTISKAKGQPREPQVYTLPPSQEEMTKNQVSLTCLVKGFYPSDIAVEWESNGQPENNYKTTPPVLDSDGSFFLYSRLTVDKSRWQEGNVFSCSVMHEALHNHYTQKSLSLSLGGGGGSGGGGSYVLTQPPSVSVAPGKTARITCGGNNLESKIVSWYQQKPGQAPVLVIFYDTDRPSGIPERFSGSNSGNTATLTISRVEAGDEADYYCQVWDSNSDHVIFGGGTKLTVLGSTSGSGKPGSGEGSTKGEVQLVESGGIVVQPGGSLRLSCAASGFTFDDYTMHWVRQAPGKGLEWVSLISWDGGSTYYADSVKGRFTISRDNSKNSLYLQMNSLRTEDTALYYCASIYDPPPGSRSALDAFDIWGQGTMVTVSSA

SEQ ID NO: 26 - protein, 706 aa, synthetic construct
  REGION 1..706: note = Anti-PD-L1-OX40 Ab-V9
QVQLVQSGAEVKKPGSSVKVSCKASGGTFRRYSISWVRQAPGQGLEWMGGIIPVFGAAKYAQKFQGRVTITADEFTSTAYMELSSLTSEDTAVYYCALSGDSDAFDIWGQGTMVTVSSASTKGPSVFPLAPCSRSTSESTAALGCLVKDYFPEPVTVSWNSGALTSGVHTFPAVLQSSGLYSLSSVVTVPSSSLGTKTYTCNVDHKPSNTKVDKRVESKYGPPCPPCPAPEFLGGPSVFLFPPKPKDTLMISRTPEVTCVVVDVSQEDPEVQFNWYVDGVEVHNAKTKPREEQFNSTYRVVSVLTVLHQDWLNGKEYKCKVSNKGLPSSIEKTISKAKGQPREPQVYTLPPSQEEMTKNQVSLTCLVKGFYPSDIAVEWESNGQPENNYKTTPPVLDSDGSFFLYSRLTVDKSRWQEGNVFSCSVMHEALHNHYTQKSLSLSLGGGGGSGGGGSYVLTQPPSVSVAPGKTARITCGGNNLESKIVSWYQQKPGQAPVLVIFYDTDRPSGIPERFSGSNSGNTATLTISRVEAGDEADYYCQVWDSNSDHVVFGGGTKLTVLGSTSGSGKPGSGEGSTKGEVQLVESGGGVVQPGGSLRLSCAASGFTFDDYTMHWVRQAPGKGLEWVSLISWDGGSTYYADSVKGRFTISRDNSKNSLYLQMNSLRTEDTALYYCASIYDPPPGSRSALDAFDIWGQGTMVTVSSA

SEQ ID NO: 27 - protein, 706 aa, synthetic construct
  REGION 1..706: note = Anti-PD-L1-OX40 Ab-V10
QVQLVQSGAEVKKPGSSVKVSCKASGGTFRRYSISWVRQAPGQGLEWMGGIIPVFGAAKYAQKFQGRVTITADEFTSTAYMELSSLTSEDTAVYYCALSGDSDAFDIWGQGTMVTVSSASTKGPSVFPLAPCSRSTSESTAALGCLVKDYFPEPVTVSWNSGALTSGVHTFPAVLQSSGLYSLSSVVTVPSSSLGTKTYTCNVDHKPSNTKVDKRVESKYGPPCPPCPAPEFLGGPSVFLFPPKPKDTLMISRTPEVTCVVVDVSQEDPEVQFNWYVDGVEVHNAKTKPREEQFNSTYRVVSVLTVLHQDWLNGKEYKCKVSNKGLPSSIEKTISKAKGQPREPQVYTLPPSQEEMTKNQVSLTCLVKGFYPSDIAVEWESNGQPENNYKTTPPVLDSDGSFFLYSRLTVDKSRWQEGNVFSCSVMHEALHNHYTQKSLSLSLGGGGGSGGGGSYVLTQPPSVSVAPGQTARITCGGNNLESKIVSWYQQKPGQAPVLVIFYDTDRPSGIPERFSGSNSGNTATLTISRVEAGDEADYYCQVWDSNSDHVVFGGGTKLTVLGSTSGSGKPGSGEGSTKGEVQLVESGGGVVQPGGSLRLSCAASGFTFDDYTMHWVRQAPGKGLEWVSLISWDGGSTYYADSVKGRFTISRDNSKNSLYLQMNSLRTEDTALYYCASIYDPPPGSRSALDAFDIWGQGTMVTVSSA

SEQ ID NO: 28 - protein, 706 aa, synthetic construct
  REGION 1..706: note = Anti-PD-L1-OX40 Ab-V11
QVQLVQSGAEVKKPGSSVKVSCKASGGTFRRYSISWVRQAPGQGLEWMGGIIPVFGAAKYAQKFQGRVTITADEFTSTAYMELSSLTSEDTAVYYCALSGDSDAFDIWGQGTMVTVSSASTKGPSVFPLAPCSRSTSESTAALGCLVKDYFPEPVTVSWNSGALTSGVHTFPAVLQSSGLYSLSSVVTVPSSSLGTKTYTCNVDHKPSNTKVDKRVESKYGPPCPPCPAPEFLGGPSVFLFPPKPKDTLMISRTPEVTCVVVDVSQEDPEVQFNWYVDGVEVHNAKTKPREEQFNSTYRVVSVLTVLHQDWLNGKEYKCKVSNKGLPSSIEKTISKAKGQPREPQVYTLPPSQEEMTKNQVSLTCLVKGFYPSDIAVEWESNGQPENNYKTTPPVLDSDGSFFLYSRLTVDKSRWQEGNVFSCSVMHEALHNHYTQKSLSLSLGGGGGSGGGGSYVLTQPPSVSVTPGETARIACGGNNLESKIVSWYQQKPGQAPVLVIFYDTDRPSGISERFSGSNSGNTATLTISRVEAGDEADYYCQVWDSNSDHVIFGGGTKLTVLGSTSGSGKPGSGEGSTKGEVQLVESGGVVVQPGGSLRLSCAASGFTFDDYTMHWVRQAPGKGLEWVSLISWDGGSTYYADSVKGRFTISRDNSKNSLYLQMNSLRTEDTALYYCASIYDPPPGSRSALDAFDIWGQGTMVTVSSA

SEQ ID NO: 29 - protein, 706 aa, synthetic construct
  REGION 1..706: note = Anti-PD-L1-OX40 Ab-V12
QVQLVQSGAEVKKPGSSVKVSCKASGGTFRRYSISWVRQAPGQGLEWMGGIIPVFGAAKYAQKFQGRVTITADEFTSTAYMELSSLTSEDTAVYYCALSGDSDAFDIWGQGTMVTVSSASTKGPSVFPLAPCSRSTSESTAALGCLVKDYFPEPVTVSWNSGALTSGVHTFPAVLQSSGLYSLSSVVTVPSSSLGTKTYTCNVDHKPSNTKVDKRVESKYGPPCPPCPAPEFLGGPSVFLFPPKPKDTLMISRTPEVTCVVVDVSQEDPEVQFNWYVDGVEVHNAKTKPREEQFNSTYRVVSVLTVLHQDWLNGKEYKCKVSNKGLPSSIEKTISKAKGQPREPQVYTLPPSQEEMTKNQVSLTCLVKGFYPSDIAVEWESNGQPENNYKTTPPVLDSDGSFFLYSRLTVDKSRWQEGNVFSCSVMHEALHNHYTQKSLSLSLGGGGGSGGGGSYVLTQPPSVSVTPGQTARIACGGNNLESKIVSWYQQKPGQAPVLVIFYDTDRPSGISERFSGSNSGNTATLTISRVEAGDEADYYCQVWDSNSDHVIFGGGTKLTVLGSTSGSGKPGSGEGSTKGEVQLVESGGVVVQPGGSLRLSCAASGFTFDDYTMHWVRQAPGKGLEWVSLISWDGGSTYYADSVKGRFTISRDNSKNSLYLQMNSLRTEDTALYYCASIYDPPPGSRSALDAFDIWGQGTMVTVSSA

SEQ ID NO: 30 - protein, 176 aa, synthetic construct
  REGION 1..176: note = Anti-PD-L1-OX40 Ab-V4
LSLGGGGGSGGGGSYVLTQPPSVSVTPGKTARIACGGNNLESKIVSWYQQKPGQAPVLVIFYDTDRPSGISERFSGSNSGNTATLTISRVEAGDEADYYCQVWDSNSDHVIFGGGTKLTVLGSTSGSGKPGSGEGSTKGEVQLVESGGVVVQPGGSLRLSCAASGFTFDDYTMHWV

SEQ ID NO: 31 - protein, 176 aa, synthetic construct
  REGION 1..176: note = Anti-PD-L1-OX40 Ab-V5
LSLGGGGGSGGGGSYELTQPPSVSVTPGQTARIACGGNNLESKIVSWYQQKPGQAPVLVIFYDTDRPSGISERFSGSNSGNTATLTISRVEAGDEADYYCQVWDSNSDHVIFGGGTKLTVLGSTSGSGKPGSGEGSTKGEVQLVESGGVVVQPGGSLRLSCAASGFTFDDYTMHWV

SEQ ID NO: 32 - protein, 176 aa, synthetic construct
  REGION 1..176: note = Anti-PD-L1-OX40 Ab-V6
LSLGGGGGSGGGGSYVLTQPPSVSVTPGETARIACGGNNLESKIVSWYQQKPGQAPVLVIFYDTDRPSGISERFSGSNSGNTATLTISRVEAGDEADYYCQVWDSNSDHVVFGGGTKLTVLGSTSGSGKPGSGEGSTKGEVQLVESGGGVVQPGGSLRLSCAASGFTFDDYTMHWV

SEQ ID NO: 33 - protein, 176 aa, synthetic construct
  REGION 1..176: note = Anti-PD-L1-OX40 Ab-V7
LSLGGGGGSGGGGSYVLTQPPSVSVTPGQTARIACGGNNLESKIVSWYQQKPGQAPVLVIFYDTDRPSGISERFSGSNSGNTATLTISRVEAGDEADYYCQVWDSNSDHVVFGGGTKLTVLGSTSGSGKPGSGEGSTKGEVQLVESGGGVVQPGGSLRLSCAASGFTFDDYTMHWV

SEQ ID NO: 34 - protein, 176 aa, synthetic construct
  REGION 1..176: note = Anti-PD-L1-OX40 Ab-V8
LSLGGGGGSGGGGSYVLTQPPSVSVAPGKTARITCGGNNLESKIVSWYQQKPGQAPVLVIFYDTDRPSGIPERFSGSNSGNTATLTISRVEAGDEADYYCQVWDSNSDHVIFGGGTKLTVLGSTSGSGKPGSGEGSTKGEVQLVESGGIVVQPGGSLRLSCAASGFTFDDYTMHWV

SEQ ID NO: 35 - protein, 176 aa, synthetic construct
  REGION 1..176: note = Anti-PD-L1-OX40 Ab-V9
LSLGGGGGSGGGGSYVLTQPPSVSVAPGKTARITCGGNNLESKIVSWYQQKPGQAPVLVIFYDTDRPSGIPERFSGSNSGNTATLTISRVEAGDEADYYCQVWDSNSDHVVFGGGTKLTVLGSTSGSGKPGSGEGSTKGEVQLVESGGGVVQPGGSLRLSCAASGFTFDDYTMHWV

SEQ ID NO: 36 - protein, 176 aa, synthetic construct
  REGION 1..176: note = Anti-PD-L1-OX40 Ab-V10
LSLGGGGGSGGGGSYVLTQPPSVSVAPGQTARITCGGNNLESKIVSWYQQKPGQAPVLVIFYDTDRPSGIPERFSGSNSGNTATLTISRVEAGDEADYYCQVWDSNSDHVVFGGGTKLTVLGSTSGSGKPGSGEGSTKGEVQLVESGGGVVQPGGSLRLSCAASGFTFDDYTMHWV

SEQ ID NO: 37 - protein, 176 aa, synthetic construct
  REGION 1..176: note = Anti-PD-L1-OX40 Ab-V11
LSLGGGGGSGGGGSYVLTQPPSVSVTPGETARIACGGNNLESKIVSWYQQKPGQAPVLVIFYDTDRPSGISERFSGSNSGNTATLTISRVEAGDEADYYCQVWDSNSDHVIFGGGTKLTVLGSTSGSGKPGSGEGSTKGEVQLVESGGVVVQPGGSLRLSCAASGFTFDDYTMHWV

SEQ ID NO: 38 - protein, 176 aa, synthetic construct
  REGION 1..176: note = Anti-PD-L1-OX40 Ab-V12
LSLGGGGGSGGGGSYVLTQPPSVSVTPGQTARIACGGNNLESKIVSWYQQKPGQAPVLVIFYDTDRPSGISERFSGSNSGNTATLTISRVEAGDEADYYCQVWDSNSDHVIFGGGTKLTVLGSTSGSGKPGSGEGSTKGEVQLVESGGVVVQPGGSLRLSCAASGFTFDDYTMHWV

SEQ ID NO: 39 - protein, 15 aa, synthetic construct
  REGION 1..15: note = linker
GGGGSGGGGSGGGGS

SEQ ID NO: 40 - protein, 19 aa, synthetic construct
  REGION 1..19: note = linker
SSGGGGSGGGGGGSSRSSL

SEQ ID NO: 41 - protein, 20 aa, synthetic construct
  REGION 1..20: note = linker
GGKGSGGKGTGGKGSGGKGS

SEQ ID NO: 42 - protein, 13 aa, synthetic construct
  REGION 1..13: note = linker
GSASAPTLFPLVS

SEQ ID NO: 43 - protein, 18 aa, synthetic construct
  REGION 1..18: note = linker
GSTSGSGKPGSGEGSTKG